European Patent Application EP 4 567 113 A1, published June 11, 2025. Title: コラーゲン産生方法. Applicant: 株式会社ＵｎｉＢｉｏ. Application WO, filed July 31, 2023. The sequence listing filed with the application follows.

SEQUENCE LISTING (27 sequences)

SEQ ID NO: 1 - DNA, 346 bp, Cauliflower mosaic virus
  source 1..346: mol_type = other DNA
tgagacttttcaacaaagggtaatatccggaaacctcctcggattccattgcccagctatctgtcactttattgtgaagatagtggaaaaggaaggtggctcctacaaatgccatcattgcgataaaggaaaggccatcgttgaagatgcctctgccgacagtggtcccaaagatggacccccacccacgaggagcatcgtggaaaaagaagacgttccaaccacgtcttcaaagcaagtggattgatgtgatatctccactgacgtaagggatgacgcacaatcccactatccttcgcaagacccttcctctatataaggaagttcatttcatttggagagaaca

SEQ ID NO: 2 - DNA, 56 bp, Tobacco mosaic virus
  source 1..56: mol_type = other DNA
acaattaccaacaacaacaaacaacaaacaacattacaattactatttacaattac

SEQ ID NO: 3 - DNA, 58 bp, Arabidopsis thaliana
  source 1..58: mol_type = other DNA
tacatcacaatcacacaaaactaacaaaagatcaaaagcaagttcttcactgttgata

SEQ ID NO: 4 - DNA, 249 bp, Arabidopsis thaliana
  source 1..249: mol_type = other DNA
tatgaagatgaagatgaaatatttggtgtgtcaaataaaaagctagcttgtgtgcttaagtttgtgtttttttcttggcttgttgtgttatgaatttgtggctttttctaatattaaatgaatgtaagatctcattataatgaataaacaaatgtttctataatccattgtgaatgttttgttggatctcttcgcatataactactgtatgtgctatggtatggactatggaatatgattaaagataag

SEQ ID NO: 5 - protein, 24 aa, Hordeum vulgare
MANKHLSLSLFLVLLGLSASLASG

SEQ ID NO: 6 - protein, 44 aa, Hordeum vulgare
MAHARVLLLALAVLATAAVAVASSSSFADSNPIRPVTDRAASTL

SEQ ID NO: 7 - protein, 139 aa, Homo sapiens
QEEGQVEGQDEDIPPITCVQNGLRYHDRDVWKPEPCRICVCDNGKVLCDDVICDETKNCPGAEVPEGECCPVCPDGSESPTDQETTGVEGPKGDTGPRGPRGPAGPPGRDGIPGQPGLPGPPGPPGPPGPPGLGGNFAP

SEQ ID NO: 8 - protein, 1442 aa, Homo sapiens
QEEGQVEGQDEDIPPITCVQNGLRYHDRDVWKPEPCRICVCDNGKVLCDDVICDETKNCPGAEVPEGECCPVCPDGSESPTDQETTGVEGPKGDTGPRGPRGPAGPPGRDGIPGQPGLPGPPGPPGPPGPPGLGGNFAPQLSYGYDEKSTGGISVPGPMGPSGPRGLPGPPGAPGPQGFQGPPGEPGEPGASGPMGPRGPPGPPGKNGDDGEAGKPGRPGERGPPGPQGARGLPGTAGLPGMKGHRGFSGLDGAKGDAGPAGPKGEPGSPGENGAPGQMGPRGLPGERGRPGAPGPAGARGNDGATGAAGPPGPTGPAGPPGFPGAVGAKGEAGPQGPRGSEGPQGVRGEPGPPGPAGAAGPAGNPGADGQPGAKGANGAPGIAGAPGFPGARGPSGPQGPGGPPGPKGNSGEPGAPGSKGDTGAKGEPGPVGVQGPPGPAGEEGKRGARGEPGPTGLPGPPGERGGPGSRGFPGADGVAGPKGPAGERGSPGPAGPKGSPGEAGRPGEAGLPGAKGLTGSPGSPGPDGKTGPPGPAGQDGRPGPPGPPGARGQAGVMGFPGPKGAAGEPGKAGERGVPGPPGAVGPAGKDGEAGAQGPPGPAGPAGERGEQGPAGSPGFQGLPGPAGPPGEAGKPGEQGVPGDLGAPGPSGARGERGFPGERGVQGPPGPAGPRGANGAPGNDGAKGDAGAPGAPGSQGAPGLQGMPGERGAAGLPGPKGDRGDAGPKGADGSPGKDGVRGLTGPIGPPGPAGAPGDKGESGPSGPAGPTGARGAPGDRGEPGPPGPAGFAGPPGADGQPGAKGEPGDAGAKGDAGPPGPAGPAGPPGPIGNVGAPGAKGARGSAGPPGATGFPGAAGRVGPPGPSGNAGPPGPPGPAGKEGGKGPRGETGPAGRPGEVGPPGPPGPAGEKGSPGADGPAGAPGTPGPQGIAGQRGVVGLPGQRGERGFPGLPGPSGEPGKQGPSGASGERGPPGPMGPPGLAGPPGESGREGAPGAEGSPGRDGSPGAKGDRGETGPAGPPGAPGAPGAPGPVGPAGKSGDRGETGPAGPTGPVGPVGARGPAGPQGPRGDKGETGEQGDRGIKGHRGFSGLQGPPGPPGSPGEQGPSGASGPAGPRGPPGSAGAPGKDGLNGLPGPIGPPGPRGRTGDAGPVGPPGPPGPPGPPGPPSAGFDFSFLPQPPQEKAHDGGRYYRADDANVVRDRDLEVDTTLKSLSQQIENIRSPEGSRKNPARTCRDLKMCHSDWKSGEYWIDPNQGCNLDAIKVFCNMETGETCVYPTQPSVAQKNWYISKNPKDKRHVWFGESMTDGFQFEYGGQGSDPADVAIQLTFLRLMSTEASQNITYHCKNSVAYMDQQTGNLKKALLLQGSNEIEIRAEGNSRFTYSVTVDGCTSHTGAWGKTVIEYKTTKTSRLPIIDVAPLDVGAPDQEFGFDVGPVCFL

SEQ ID NO: 9 - protein, 246 aa, synthetic construct
DDANVVRDRDLEVDTTLKSLSQQIENIRSPEGSRKNPARTCRDLKMCHSDWKSGEYWIDPNQGCNLDAIKVFCNMETGETCVYPTQPSVAQKNWYISKNPKDKRHVWFGESMTDGFQFEYGGQGSDPADVAIQLTFLRLMSTEASQNITYHCKNSVAYMDQQTGNLKKALLLQGSNEIEIRAEGNSRFTYSVTVDGCTSHTGAWGKTVIEYKTTKTSRLPIIDVAPLDVGAPDQEFGFDVGPVCFL

SEQ ID NO: 10 - protein, 57 aa, synthetic construct
QSLQEETVRKGPAGDRGPRGERGPPGPPGRDGEDGPTGPPGPPGPPGPPGLGGNFAA

SEQ ID NO: 11 - protein, 1344 aa, Homo sapiens
QSLQEETVRKGPAGDRGPRGERGPPGPPGRDGEDGPTGPPGPPGPPGPPGLGGNFAAQYDGKGVGLGPGPMGLMGPRGPPGAAGAPGPQGFQGPAGEPGEPGQTGPAGARGPAGPPGKAGEDGHPGKPGRPGERGVVGPQGARGFPGTPGLPGFKGIRGHNGLDGLKGQPGAPGVKGEPGAPGENGTPGQTGARGLPGERGRVGAPGPAGARGSDGSVGPVGPAGPIGSAGPPGFPGAPGPKGEIGAVGNAGPAGPAGPRGEVGLPGLSGPVGPPGNPGANGLTGAKGAAGLPGVAGAPGLPGPRGIPGPVGAAGATGARGLVGEPGPAGSKGESGNKGEPGSAGPQGPPGPSGEEGKRGPNGEAGSAGPPGPPGLRGSPGSRGLPGADGRAGVMGPPGSRGASGPAGVRGPNGDAGRPGEPGLMGPRGLPGSPGNIGPAGKEGPVGLPGIDGRPGPIGPAGARGEPGNIGFPGPKGPTGDPGKNGDKGHAGLAGARGAPGPDGNNGAQGPPGPQGVQGGKGEQGPPGPPGFQGLPGPSGPAGEVGKPGERGLHGEFGLPGPAGPRGERGPPGESGAAGPTGPIGSRGPSGPPGPDGNKGEPGVVGAVGTAGPSGPSGLPGERGAAGIPGGKGEKGEPGLRGEIGNPGRDGARGAPGAVGAPGPAGATGDRGEAGAAGPAGPAGPRGSPGERGEVGPAGPNGFAGPAGAAGQPGAKGERGAKGPKGENGVVGPTGPVGAAGPAGPNGPPGPAGSRGDGGPPGMTGFPGAAGRTGPPGPSGISGPPGPPGPAGKEGLRGPRGDQGPVGRTGEVGAVGPPGFAGEKGPSGEAGTAGPPGTPGPQGLLGAPGILGLPGSRGERGLPGVAGAVGEPGPLGIAGPPGARGPPGAVGSPGVNGAPGEAGRDGNPGNDGPPGRDGQPGHKGERGYPGNIGPVGAAGAPGPHGPVGPAGKHGNRGETGPSGPVGPAGAVGPRGPSGPQGIRGDKGEPGEKGPRGLPGLKGHNGLQGLPGIAGHHGDQGAPGSVGPAGPRGPAGPSGPAGKDGRTGHPGTVGPAGIRGPQGHQGPAGPPGPPGPPGPPGVSGGGYDFGYDGDFYRADQPRSAPSLRPKDYEVDATLKSLNNQIETLLTPEGSRKNPARTCRDLRLSHPEWSSGYYWIDPNQGCTMDAIKVYCDFSTGETCIRAQPENIPAKNWYRSSKDKKHVWLGETINAGSQFEYNVEGVTSKEMATQLAFMRLLANYASQNITYHCKNSIAYMDEETGNLKKAVILQGSNDVELVAEGNSRFTYTVLVDGCSKKTNEWGKTIIEYKTNKPSRLPFLDIAPLDIGGADQEFFVDIGPVCFK

SEQ ID NO: 12 - protein, 247 aa, synthetic construct
DQPRSAPSLRPKDYEVDATLKSLNNQIETLLTPEGSRKNPARTCRDLRLSHPEWSSGYYWIDPNQGCTMDAIKVYCDFSTGETCIRAQPENIPAKNWYRSSKDKKHVWLGETINAGSQFEYNVEGVTSKEMATQLAFMRLLANYASQNITYHCKNSIAYMDEETGNLKKAVILQGSNDVELVAEGNSRFTYTVLVDGCSKKTNEWGKTIIEYKTNKPSRLPFLDIAPLDIGGADQEFFVDIGPVCFK

SEQ ID NO: 13 - protein, 237 aa, synthetic construct
SKGEELFTGVVPILVELDGDVNGHKFSVSGEGEGDATYGKLTLKFICTTGKLPVPWPTLVTTFSYGVQCFSRYPDHMKQHDFFKSAMPEGYVQERTIFFKDDGNYKTRAEVKFEGDTLVNRIELKGIDFKEDGNILGHKLEYNYNSHNVYIMADKQKNGIKVNFKIRHNIEDGSVQLADHYQQNTPIGDGPVLLPDNHYLSTQSALSKDPNEKRDHMVLLEFVTAAGITHGMDELYK

SEQ ID NO: 14 - protein, 217 aa, synthetic construct
SPILGYWKIKGLVQPTRLLLEYLEEKYEEHLYERDEGDKWRNKKFELGLEFPNLPYYIDGDVKLTQSMAIIRYIADKHNMLGGCPKERAEISMLEGAVLDIRYGVSRIAYSKDFETLKVDFLSKLPEMLKMFEDRLCHKTYLNGDHVTHPDFMLYDALDVVLYMDPMCLDAFPKLVCFKKRIEAIPQIDKYLKSSKYIAWPLQGWQATFGGGDHPPK

SEQ ID NO: 15 - protein, 382 aa, Escherichia coli
KIEEGKLVIWINGDKGYNGLAEVGKKFEKDTGIKVTVEHPDKLEEKFPQVAATGDGPDIIFWAHDRFGGYAQSGLLAEITPDKAFQDKLYPFTWDAVRYNGKLIAYPIAVEALSLIYNKDLLPNPPKTWEEIPALDKELKAKGKSALMFNLQEPYFTWPLIAADGGYAFKYENGKYDIKDVGVDNAGAKAGLTFLVDLIKNKHMNADTDYSIAEAAFNKGETAMTINGPWAWSNIDTSKVNYGVTVLPTFKGQPSKPFVGVLSAGINAASPNKELAKEFLENYLLTDEGLEAVNKDKPLGAVALKSYEEELVKDPRIAATMENAQKGEIMPNIPQMSAFWYAVRTAVINAASGRQTVDEALKDAQTNSSSNNNNNNNNNNLG

SEQ ID NO: 16 - protein, 12 aa, synthetic construct
HNHNHNHNHNHN

SEQ ID NO: 17 - protein, 517 aa, Homo sapiens
HPGFFTSIGQMTDLIHTEKDLVTSLKDYIKAEEDKLEQIKKWAEKLDRLTSTATKDPEGFVGHPVNAFKLMKRLNTEWSELENLVLKDMSDGFISNLTIQRQYFPNDEDQVGAAKALLRLQDTYNLDTDTISKGNLPGVKHKSFLTAEDCFELGKVAYTEADYYHTELWMEQALRQLDEGEISTIDKVSVLDYLSYAVYQQGDLDKALLLTKKLLELDPEHQRANGNLKYFEYIMAKEKDVNKSASDDQSDQKTTPKKKGVAVDYLPERQKYEMLCRGEGIKMTPRRQKKLFCRYHDGNRNPKFILAPAKQEDEWDKPRIIRFHDIISDAEIEIVKDLAKPRLRRATISNPITGDLETVHYRISKSAWLSGYENPVVSRINMRIQDLTGLDVSTAEELQVANYGVGGQYEPHFDFARKDEPDAFKELGTGNRIATWLFYMSDVSAGGATVFPEVGASVWPKKGTAVFWYNLFASGEGDYSTRHAACPVLVGNKWVSNKWLHERGQEFRRPCTLSELE

SEQ ID NO: 18 - protein, 543 aa, Caenorhabditis elegans
DLFTSIADMQNLLETERNIPKILDKYIHDEEERLVQLKKLSEEYSKKNEISIENGLKDITNPINAFLLIKRKIFDWKEIESKMNANKAGNVVSSITDDSYGVRYPTADDLSGAAIGLLRLQDTYRLDTKDLADGKIYADQGNYTFSAKDCFEIARAAYNEHDFYHTVMWMEEAQRRLGDEVEPTVEVEDILEYLAFALYKQNNLKHALKLTEELYKMNPTHPRAKGNVKWYEDLLEQEGVRRSDMRKNLPPIQNRRPDSVLGNTERTMYEALCRNEVPVSQKDISRLYCYYKRDRPFLVYAPIKVEIKRFNPLAVLFKDVISDDEVAAIQELAKPKLARATVHDSVTGKLVTATYRISKSAWLKEWEGDVVETVNKRIGYMTNLEMETAEELQIANYGIGGHYDPHFDHAKKEESKSFESLGTGNRIATVLFYMSQPSHGGGTVFTEAKSTILPTKNDALFWYNLYKQGDGNPDTRHAACPVLVGIKWVSNKWIHEKGNEFRRPCGLKSSDYERFVGDLGYGPEPRNAPNVSPNLAKDVWETL

SEQ ID NO: 19 - protein, 487 aa, Homo sapiens
DAPEEEDHVLVLRKSNFAEALAAHKYLLVEFYAPWCGHCKALAPEYAKAAGKLKAEGSEIRLAKVDATEESDLAQQYGVRGYPTIKFFRNGDTASPKEYTAGREADDIVNWLKKRTGPAATTLPDGAAAESLVESSEVAVIGFFKDVESDSAKQFLQAAEAIDDIPFGITSNSDVFSKYQLDKDGVVLFKKFDEGRNNFEGEVTKENLLDFIKHNQLPLVIEFTEQTAPKIFGGEIKTHILLFLPKSVSDYDGKLSNFKTAAESFKGKILFIFIDSDHTDNQRILEFFGLKKEECPAVRLITLEEEMTKYKPESEELTAERITEFCHRFLEGKIKPHLMSQELPEDWDKQPVKVLVGKNFEDVAFDEKKNVFVEFYAPWCGHCKQLAPIWDKLGETYKDHENIVIAKMDSTANEVEAVKVHSFPTLKFFPASADRTVIDYNGERTLDGFKKFLESGGQDGAGDDDDLEDLEEAEEPDMEEDDDQKAV

SEQ ID NO: 20 - protein, 490 aa, Mus musculus
DALEEEDNVLVLKKSNFEEALAAHKYLLVEFYAPWCGHCKALAPEYAKAAAKLKAEGSEIRLAKVDATEESDLAQQYGVRGYPTIKFFKNGDTASPKEYTAGREADDIVNWLKKRTGPAATTLSDTAAAESLVDSSEVTVIGFFKDVESDSAKQFLLAAEAIDDIPFGITSNSGVFSKYQLDKDGVVLFKKFDEGRNNFEGEITKEKLLDFIKHNQLPLVIEFTEQTAPKIFGGEIKTHILLFLPKSVSDYDGKLSSFKRAAEGFKGKILFIFIDSDHTDNQRILEFFGLKKEECPAVRLITLEEEMTKYKPESDELTAEKITEFCHRFLEGKIKPHLMSQEVPEDWDKQPVKVLVGANFEEVAFDEKKNVFVEFYAPWCGHCKQLAPIWDKLGETYKDHENIIIAKMDSTANEVEAVKVHSFPTLKFFPASADRTVIDYNGERTLDGFKKFLESGGQDGAGDDEDLDLEEALEPDMEEDDDQKAVKDEL

SEQ ID NO: 21 - protein, 714 aa, Homo sapiens
SDRPRGRDPVNPEKLLVITVATAETEGYLRFLRSAEFFNYTVRTLGLGEEWRGGDVARTVGGGQKVRWLKKEMEKYADREDMIIMFVDSYDVILAGSPTELLKKFVQSGSRLLFSAESFCWPEWGLAEQYPEVGTGKRFLNSGGFIGFATTIHQIVRQWKYKDDDDDQLFYTRLYLDPGLREKLSLNLDHKSRIFQNLNGALDEVVLKFDRNRVRIRNVAYDTLPIVVHGNGPTKLQLNYLGNYVPNGWTPEGGCGFCNQDRRTLPGGQPPPRVFLAVFVEQPTPFLPRFLQRLLLLDYPPDRVTLFLHNNEVFHEPHIADSWPQLQDHFSAVKLVGPEEALSPGEARDMAMDLCRQDPECEFYFSLDADAVLTNLQTLRILIEENRKVIAPMLSRHGKLWSNFWGALSPDEYYARSEDYVELVQRKRVGVWNVPYISQAYVIRGDTLRMELPQRDVFSGSDTDPDMAFCKSFRDKGIFLHLSNQHEFGRLLATSRYDTEHLHPDLWQIFDNPVDWKEQYIHENYSRALEGEGIVEQPCPDVYWFPLLSEQMCDELVAEMEHYGQWSGGRHEDSRLAGGYENVPTVDIHMKQVGYEDQWLQLLRTYVGPMTESLFPGYHTKARAVMNFVVRYRPDEQPSLRPHHDSSTFTLNVALNHKGLDYEGGGCRFLRYDCVISSPRKGWALLHPGRLTHYHEGLPTTWGTRYIMVSFVDP

SEQ ID NO: 22 - protein, 610 aa, Homo sapiens
AATSRPERVWPDGVIPFVIGGNFTGSQRAVFRQAMRHWEKHTCVTFLERTDEDSYIVFTYRPCGCCSYVGRRGGGPQAISIGKNCDKFGIVVHELGHVVGFWHEHTRPDRDRHVSIVRENIQPGQEYNFLKMEPQEVESLGETYDFDSIMHYARNTFSRGIFLDTIVPKYEVNGVKPPIGQRTRLSKGDIAQARKLYKCPACGETLQDSTGNFSSPEYPNGYSAHMHCVWRISVTPGEKIILNFTSLDLYRSRLCWYDYVEVRDGFWRKAPLRGRFCGSKLPEPIVSTDSRLWVEFRSSSNWVGKGFFAVYEAICGGDVKKDYGHIQSPNYPDDYRPSKVCIWRIQVSEGFHVGLTFQSFEIERHDSCAYDYLEVRDGHSESSTLIGRYCGYEKPDDIKSTSSRLWLKFVSDGSINKAGFAVNFFKEVDECSRPNRGGCEQRCLNTLGSYKCSCDPGYELAPDKRRCEAACGGFLTKLNGSITSPGWPKEYPPNKNCIWQLVAPTQYRISLQFDFFETEGNDVCKYDFVEVRSGLTADSKLHGKFCGSEKPEVITSQYNNMRVEFKSDNTVSKKGFKAHFFSEKRPALQPPRGRPHQLKFRVQKRNRTPQ

SEQ ID NO: 23 - protein, 172 aa, Tomato bushy stunt virus
MERAIQGNDAREQANSERWDGGSGSSTSPFQLPDESPSWTEWRLHNDETNSNQDNPLGFKESWGFGKVVFKRYLRYERTETSLHRVLGSWTGDSVNYAASRFFGVNQIGCTYSIRFRGVSVTISGGSRTLQHLCEMAIRSKQELLQLTPVEVESNVSRGCPEGVETFEEESE

SEQ ID NO: 24 - protein, 8 aa, synthetic construct
LEVLFQGP

SEQ ID NO: 25-26 - skipped (2 entries)

SEQ ID NO: 27 - protein, 5 aa, synthetic construct
DDDDK